European Patent Application EP 4 282 879 A2, published November 29, 2023. Title: USE OF FERTILE TRANSGENIC ANIMALS FOR PRODUCING ANTIBODIES BEARING HUMAN VARIABLE REGIONS. Applicant: Kymab Limited. The sequence listing filed with the application follows.

SEQUENCE LISTING (9 sequences)

SEQ ID NO: 1 - DNA, 2256 bp, Rattus norvegicus
  source 1..2256: mol_type = genomic DNA
atgttatctctgacctggggtatgaagctagtggaaagatctgtggtccccagggtcctcctcttgctctttgcactctggctgctcctcctggttccagtccggtgttctgaaggccaccccacttggcgctacatctcatcagaggtggttattcctcggaaggagatctaccacagcaaaggaattcaaacacaaggacggctctcctatagcttgcgttttaggggccagagacatatcatccacctgcgaagaaagacactaatttggcccagacacttgttgctgacaactcaggatgaccaaggagccttacagatggattacccttttttccctgtagattgttactattttggctacctagagggaatccctcaatccatggtcactgtgaatacttgctatggaggcctggaagggatcatgatgttggatgaccttgcctatgaaatcaaacccctcaacgattcacaggggtttgaacacattgtttctcagatagtatcagagcctgatgtaacagggcctacaaatacatggaaacgcttgaaccttaatacaggtcctcccttatccaggacagagtatgccaatggaactcccagaatgtctagtaagaactacgcttcacatccagctgctataaaaggccaattccaagcaactaattctatatataaggaaagcaacaatattgatactgcggccaggtatttgtttgagctccttagtataacggacagctttctgatcactattcatatgcggtactatgctattctcttaactgtgtttaccgagagcgatccatttgcactagagtatacggtaccagggggctctatttataactattatgtgtctaacttttttaatcggttgaggcctgatgcatcaaccgtacttaataaagatgggccctcggataacgactttcatccagttgaacagagtttatgtactcccgcaggcctgacgattgttggtcaacacagacgaagttttctagctctatctgttatgatcaccaatcgtattgcgatgtctttaggtataaaagctgatgatgagacttactgcatctgccacagaaggaccacttgcattatgtacaaaaaccctgaaataacagatgctttcagcaattgctcccttgtgcagataaaccagatactgaatacccctggtacaatgtcatgccttttctatgaccaccatgtttatcataatataacaaaaacctacaggttttgtggaaacttcaagatagatatcggtgagcagtgtgactgtggctcacataaggcatgttacgcagatccctgctgcggaagtaattgcaagttaactgctggtagcatttgtgataaagaattatgctgtgcaaactgcacctacagtccttctgggacactctgcagaccgatccagaacatatgtgatcttccagaatactgtagtgggaataatatcttttgccctgcagacacttatctgcaagatgggacgccatgctcagaagaggggtactgctataaaggcaactgcacagatcgcagtgtgcagtgcaaggaaatctttggtatgaatgctaagggtgctaatatcaagtgctatgacatcaacaaacaacggtttcgatttgggcactgcactagagcacaagagagcctcatgtttaatgcttgctctgatcatgataaactgtgtggaaggctgcagtgtaccaacgtcaccaatcttccattcctgcaggaacatgtttcattccatcaatcggttatctctgggtttacctgctttgggcttgatgaacatcgtgggacagaaacaacggatgctgggctggtgaaacatggtaccccttgctcccaaactaacttctgcgatcgaggagcttgcaatggaagtttatctcggttggattatgactgcaccccagaaaaatgcaattttagaggagtgtgtaataatcatcggcattgccattgtcatttaggttggaaacctcctctgtgcagagaggaggggcctagcgggagcacggacagtgggtcccctccgaaggaaaggcgcacaataaaacagagcagagaaccactgttatatttaagaatgctctttggtcgtctttatttattcattgtctcgctgctctttggagtggccactcgcgcaggagttattaaggtctttaagtttgaagacttgcaagctgctctgcgggctgcacaagccaaggcgacttaa

SEQ ID NO: 2 - DNA, 2196 bp, Oryctolagus cuniculus
  source 1..2196: mol_type = genomic DNA
atggtgctggcagaaggacaggtcacgctgctcctgcttgggctctgggtgctcctagacccaggtcagtgttccccaggccgcccctcctggcgctatgtctcatctgaggtggtgattcctcggaaggagctgcaccagggcagaggtgttcaggtagcaggctggctctccatcagcctgcactttgggggccaaagacacgtcatctgtatgcggagcaagaagcttatttgggccagacacctgatgatgatgacccaagatgaccaaggagcgttgcagatggactatccttacattcctacagactgttactacctcggccacctggaagacattcctctgtccaccgtcaccattgacacgtgctatgggggcctggaaggcatcatgaagttggatgacctcgcctatgaaatcaaacccctcaaggactccaacacatttgaacacgttgtgtctcagatcgtggccgaccgcaatgccacgggacccatgtacagactggaacacgaggacgattttgaccccttcttctccgaggtaaacagtagtgtggctcccaagctctctagtttcaaccacatgtaccacatggcccaattgaaaggtcaaattcaaatagcccacgaaatgtatacggtactcaacaatatttcaaaatgcatccaattttcaataaacatgtttagtattattgacagttttctgagaggaattggctttaggcactatattgctctcctaaacatatacaaccagcaagagccagtcgttatgaatgattttcgggttcctggcggtccaatccatgcttattataaagcgaattttcatgacatctaccgcccttctccatcgacattgattacaagaaatgcaccaaatgatgattaccaagaacccgctaggtatggcacctgtggccatcataacttgcttatcattggttcccagggcagacattatctcctgttggctattttaactacacataaaattgcacgacagatagggttagcatatgactacagtgtctgtgtgtgccagagaagagcaacctgcttgatgaggaaattccctgaaatgacagactcgttcagtaactgctcttttgtccatacacaacatatagtttcaaacagatatatttttacatgctattacttcacagataggacgtacatgaataaaaccctgatacagacgcgctgtggaaactttttagtggaagaaagggagcaatgtgattgtggctccttcaagcattgttatgccaatgcatgctgtcaaagcgactgtcgcttcacacctggaagtatttgtgataaacaacaatgctgcacaaactgcacctactcccccacttcaaccctctgcagacctgtcatgaacatatgtgatcttccagagtactgtggggggtccacctacacatgccctgaaaatttttatttgcaagacggaaccccgtgcactgaagatggttactgctacagagggaactgctctgaccccactatgcactgcaaggagatctttggtcaaagtgctgagaatggtcctgcggattgctatgccataaatctcaacaccttccgatttggacattgtagaagagagcaacatcagaacgtttaccatgcttgtgctgcacaagacaaggagtgtggaaggctacagtgcatcaatgtcacccagcttcctcagttgcaggatcatgtttcattccatcagtctgtgtacaatgagttcacctgttttggactggatgaacaccggtcaacaggatcaactgatgctggacgtgtgagagatggtactccctgtggggaaggacttttctgtcttgagagcagatgcaacatgactatgcttaacctgcattacgactgtttccctgagaagtgcagttttagaggactttgcaacaataacaagaattgccactgccatgttggctgggaccccccactgtgcctgagtccgggtgctggtgggagctcacaaagcgggccccctccaaggagaatgcgcacagtcacagatagcatggagccaattctttatttaagagtggtctttgctcgtgtttattgttttatttttgcactgctctttggggtagccactaatgtgcgaacgattaagactaccattgtccaggaacaaacagttaatgagccacagtaa

SEQ ID NO: 3 - DNA, 2265 bp, Mus musculus
  source 1..2265: mol_type = genomic DNA
atgttatctctgacctggggcatgaggctagtggaaagacctgtggtccccagggtcctcctcttgctatttgcactctggctgctcctcctggttccagtctggtgttctcaaggccatcccacttggcgttacatctcatcggaggtggttattcctcggaaggagatctaccataccaaaggacttcaagcacaaagactgctctcgtatagcttgcgttttcggggccagagacatatcatccacctgcggagaaagacactcatttggcccagacacttgttgctgacaactcaagatgaccaaggagccttacagatggagtaccccttttttcctgtagattgttactatattggctacctggaggggatcctgcaatccatggtcactgtggatacttgttatgggggcctgtcaggggtcataaagttggataaccttacctatgaaatcaaacccctcaatgattcacagagctttgaacaccttgtttctcagatagtatctgagtctgatgacacagggcctatgaatgcatggaagcactggagccataatacaggttctccctcctccagattggaatatgcagatggagctcccagactatctagtaagaattacgctacacatccagctgctataaaaggccactttcaagcaacccattctgtatatagtgcttctggaggtgacaaactttcatctactgttgagtatttgtttaaagtcattagtttaatggacacctatctgaccaatcttcatatgcggtactatgtctttctcatgactgtgtataccgaggctgatccattttcacaagattttcgagttccaggagggcaggctcatactttctatgagagagtattttatgctcattttaggcctgatgcaggagctataattaacaagaattcgccaggagatgatgctgttaatccagctgagaggagtatatgttctccctcagccctaatttgtcttggtcaacatggtcgaaatcctttatttttatctattataataaccaatcgtgttggaaggagtttaggcctaaaacatgatgaggggtactgtatctgccagagaaggaacacctgcatcatgttcaaaaatcctcaattaacagatgctttcagcaattgttcccttgcagagataagcaacatacttaatactcctgatctgatgccatgtcttttctatgaccgtcatgtttattataatacatcattgacttataagttttgtggaaacttcaaagtagataacaatgagcagtgtgactgtggctcccaaaaggcatgttattcagatccctgctgtggaaatgattgcaggttaacacctggtagcatttgtgataaagaattatgctgtgcaaattgcacttacagtccttctgggacactctgcagacctatccagaacatatgtgatcttccagagtactgtagtggctctaagttcatttgcccagatgacacttatctgcaagatgggacaccatgctcagaagagggttactgctataaaggtaactgcactgatcgcaacatacaatgcatggaaatctttggtgtaagtgctaagaatgctaatattaagtgctatgacatcaacaaacaacggtttcgatttgggcattgtactagagcagaagaaagcctcacattcaatgcttgtgctgatcaggacaagctgtgtggaaggttgcagtgtaccaatgtcaccaatcttccatttttgcaagaacatgtttcattccatcaatcggttatctctggggttacctgctttgggcttgatgaacatcgtgggacagaaacagcagatgctggattggtgagacatggtaccccgtgttcaaggggtaagttctgtgatcgaggagcttgcaatggaagtttatctcgtttgggttatgactgcaccccagaaaaatgcaatttcagaggagtgtgtaacaatcgtcggaattgccattgccattttggttggagccctccaaagtgcaaagaagagggacacagtgggagcatagacagtgggtcccctccggttcaaaggcgcataataaaacagaacctagagccagtagtgtatttaagaatactctttggtcgtatttacttcctctttgttgcactgctctttggcattgccactcgtgtaggagttactaagatatttaggtttgaagacttgcaagctgctttacgttcttggcaagaacaagcaaaggacaagtaa

SEQ ID NO: 4 - DNA, 2271 bp, Mus musculus
  source 1..2271: mol_type = genomic DNA
atgttatctctgacctggggcatgaggctagtggaaagacctgtggtccccagggtcctcctcttgctatttgcactctggctgctcctcctggttccagtctggtgttctcaaggccatcctacttggcgttacatctcatcggaggtggttattcctcggaaggagatctaccataccaaaggacttcaagcacaaagactgctctcatatagcttgcattttcggggccagagacatatcatccacctgcggagaaagacactcatttggcccagacacttgttgctgacaactcaagatgaccaaggagccttacagatggattaccccttttttcctgtagattgttactatattggctacctggaggggatcccacaatccatggtcactgtggatacttgttatgggggcctgtcaggggtcatgaagttagatgaccttacctatgaaatcaaacccctcaatgattcacagagctttgaacaccttgtttctcagatagtatctgagtctgatgacacagggcctatgaatgcatggaagcactggagccataatacaggttctccctcctccagattggaatatgcagatggagctcccagaatatctagtaagaactacgctacacatccagctgctataaaaggccactttcaagcaaccaattctgtatataattctgctgcaggtgacaaactttcatctactgttgggtatttgtttcaagtcattagtttaatggacacctatctgaccaatcttcatatgcggtactatgtctttctcatgactgtgtacaccaattctgatccatttcgacttgagtttgcagttccaggagggtcggcttataattactatgtgtcagtcttttataataaatttaagcctgatgcaggagttttacttaataagtatgggccacaagataaccaggttaatccagctgagaggagtatatgttcttccttagccctaatttgtattggtaaatatgatcgaaatcctttatttttatctcctataataaccaatcgtgttggaaggagtttaggcttaaaatatgatgaggggtactgtgtctgccagagaaggaacacctgcattatgttcagacatcctcaattaacagatgctttcagcaattgttcccttgcagagataagcaacatacttaatactcctggtctgatgccatgtcttttctatgaccgtcatgtttattataatacatcattgacttataagttttgtggaaacttcaaagtagataacgatgagcagtgtgactgtggctcccaaaaggcatgttattcagatccctgctgtggaaatgattgcaggttaacacctggtagcatttgtgataaagaattatgctgtgcaaattgcacttacagtccttctgggacactctgcagacctatccagaacatatgtgatcttccagagtactgtaatgggactaaatacatttgcccagatgacacttatctgcaagatgggacaccatgctcagaagatggttactgctataaaggtaactgcactgatcgcaacatacaatgcatggaaatctttggtgtaagtgctaagaatgctaatattaagtgctatgacatcaacaaacaacggtttcgatttgggcattgtactagagcagaagaaagcctcacattcaatgcttgtgctgatcaggacaagctgtgtggaaggttgcagtgtaccaatgtcaccaatcttccatatttgcaagaacatgtttcattccatcaatcgattatctctgggtttacctgctttgggcttgatgaacatcgtgggacagaaacaacagatgctggaatggtgagacatggtaccccctgctccaaaagtaagttctgtgatcaaggagcttgcagtggaagtttatctcatttgggttatgactgcaccccagaaaaatgcagttttagaggagtgtgtaacaatcatcggaattgccattgtcattttggttggaagcctccagagtgcaaagaagagggactaagtgggagcatagacagtgggtcccctccagttcaaaggcacacaataaaacaaaaacaagagccagtggtgtatttaagaatactctttggtcgtatttacttcctctttgttgcactgctctttggcattgccactcgtgtaggagttactaagatttttagatttgaagacttgcaagctactttacgttctgggcaaggaccagcaagggacaagccaaagtaa

SEQ ID NO: 5 - DNA, 200 bp, synthetic construct
  misc_feature 1..200: note = 5' Homology Arm:
  source 1..200: mol_type = other DNA
tatgttgatggatttccatatattaaaccatccctgcatccctgggatgaagcctacttggtcatgatagacgattgttttgatgtgttcttggattcagttagtgagaaatatattgagtatttttacatcgatattcataagggaaattggtctgaagttctctttctttgttgggtctttatgtggtttagttatca

SEQ ID NO: 6 - DNA, 204 bp, synthetic construct
  misc_feature 1..204: note = 3' Homology Arm:
  source 1..204: mol_type = other DNA
tgattccaccagaggttcttttatccttgagaagagtttttgctatcctaggttttttgttattccacatgaatttgcagattgctctttctaattccttgaagaattgagttggaatttgatggggattgcattaaatctgtagattccttttggcaagacagccatttttacaatgttaatcctgccaatccatgagcatgg

SEQ ID NO: 7 - DNA, 304 bp, synthetic construct
  misc_feature 1..304: note = 5' Homology Arm:
  source 1..304: mol_type = other DNA
tttatgtactataccatctcagaaagtcaggttagtctcactagcatcgtaaaagctctgtctgggcttttccatctgctctgctttttgtctctgtgtctaaaaatatataaaccaatgttgtccagccaaaaaaaaaaaattaaagagcaaaaggaggtaaaatggatacaaattggaaaagaagaaatcaaaatatcactacttgaagatagtataatatatttaactgaccacaaaaattccaccagaaaactcctaaacctgataaacaaactcagaaaaatggctagatataaactta

SEQ ID NO: 8 - DNA, 315 bp, synthetic construct
  misc_feature 1..315: note = 3' Homology Arm:
  source 1..315: mol_type = other DNA
acccatagagagaaaacaggtgagttagtgcattaaaggggctgagcagggagttctcatcgctccccagcaccagaaataagagcctctccggagctgctgggacatggaatgcagatgattcggaccatcagccccacagagacctttcccactctggctcagaaagaggcactggaccacagttggagaggagaatcgaaagctgatatctctgtattcacttagcctgttacccacccatgcacccaagtccaaggtgggagaaacactgagggtctaaacacagccccagagcaactgccagtattaaat

SEQ ID NO: 9 - DNA, 365 bp, synthetic construct
  misc_feature 1..365: note = IgH BAC Homology Arm:
  source 1..365: mol_type = other DNA
attcaggcagttaattgttgggttcatgttttacaactaaagaataaattcaggccagatgcagtggatcatcgctataatcacaccactttcagaagcaaaaatgagggaaatcccgtgagacgaggcaatcgaagccaacctgagcaacataaagagatgctatttctctgaaaaaatattttaaagaataagcaggtgaggggtggcgttcccctctacttctagatactcaggaagcaaagatgggaagattatgtgagccaggtgttcaaaattacagtgagctttgatcatacaactgttcttcaaactgtgcaacagggtgagagcctgtctctaaaaacaaataaaaaagaatcaat